European Patent Application EP 4 509 139 A1, published February 19, 2025. Title: CONJUGATE AND COMPOSITION AS WELL AS PREPARATION METHOD THEREFOR AND USE THEREOF. Applicant: SUZHOU RIBO LIFE SCIENCE CO., LTD. The sequence listing filed with the application follows.

SEQUENCE LISTING (54 sequences)

SEQ ID NO: 1 - RNA, 21 nt, synthetic construct
  source 1..21: mol_type = other RNA
ctgcttcagacgtgttagctt

SEQ ID NO: 2 - RNA, 22 nt, synthetic construct
  source 1..22: mol_type = other RNA
ctgagttcagacgtgttgctct

SEQ ID NO: 3 - RNA, 32 nt, synthetic construct
  source 1..32: mol_type = other RNA
tctatggctgccgatctggtctccatgtacgt

SEQ ID NO: 4 - RNA, 21 nt, synthetic construct
  source 1..21: mol_type = other RNA
  misc_feature 13: note = is T, C, or G; or a motif consisting of two of T, C, or G
  misc_feature 16: note = is T, CT, or TT
  misc_feature 21: note = is T, TT, or TTX, wherein X is a motif consisting of 1-15 nucleotides
  misc_feature 1: note = is CT, TC or AC
nggagttcannnntgngctcn

SEQ ID NO: 5 - RNA, 24 nt, synthetic construct
  source 1..24: mol_type = other RNA
ctggagttcagacgtgttgctctt

SEQ ID NO: 6 - RNA, 24 nt, synthetic construct
  source 1..24: mol_type = other RNA
ctggagttcagacgttgtgctctt

SEQ ID NO: 7 - RNA, 24 nt, synthetic construct
  source 1..24: mol_type = other RNA
ctggagttcagaccgtgtgctctt

SEQ ID NO: 8 - RNA, 23 nt, synthetic construct
  source 1..23: mol_type = other RNA
ctggagttcagacgtgttgctct

SEQ ID NO: 9 - RNA, 24 nt, synthetic construct
  source 1..24: mol_type = other RNA
acggagttcagacgtgttgctctt

SEQ ID NO: 10 - RNA, 24 nt, synthetic construct
  source 1..24: mol_type = other RNA
ctggagttcactactgttgctctt

SEQ ID NO: 11 - RNA, 24 nt, synthetic construct
  source 1..24: mol_type = other RNA
ctggagttcagttgtgttgctctt

SEQ ID NO: 12 - RNA, 32 nt, synthetic construct
  source 1..32: mol_type = other RNA
ctggagttcagacgtgttgctcttccgatctc

SEQ ID NO: 13 - RNA, 32 nt, synthetic construct
  source 1..32: mol_type = other RNA
ctggagttcagacgttgtgctcttccgatctc

SEQ ID NO: 14 - RNA, 32 nt, synthetic construct
  source 1..32: mol_type = other RNA
ctggagttcagaccgtgtgctcttccgatctc

SEQ ID NO: 15 - RNA, 32 nt, synthetic construct; identical to SEQ ID NO: 12
  source 1..32: mol_type = other RNA

SEQ ID NO: 16 - RNA, 24 nt, synthetic construct
  source 1..24: mol_type = other RNA
ctggagttcagacgtgttgctctt

SEQ ID NO: 17 - RNA, 32 nt, synthetic construct; identical to SEQ ID NO: 13
  source 1..32: mol_type = other RNA

SEQ ID NO: 18 - RNA, 24 nt, synthetic construct
  source 1..24: mol_type = other RNA
ctggagttcagacgttgtgctctt

SEQ ID NO: 19 - RNA, 32 nt, synthetic construct; identical to SEQ ID NO: 14
  source 1..32: mol_type = other RNA

SEQ ID NO: 20 - RNA, 24 nt, synthetic construct
  source 1..24: mol_type = other RNA
ctggagttcagaccgtgtgctctt

SEQ ID NO: 21 - RNA, 32 nt, synthetic construct; identical to SEQ ID NO: 12
  source 1..32: mol_type = other RNA

SEQ ID NO: 22 - RNA, 24 nt, synthetic construct
  source 1..24: mol_type = other RNA
ctggagttcagacgtgttgctctt

SEQ ID NO: 23 - RNA, 32 nt, synthetic construct; identical to SEQ ID NO: 13
  source 1..32: mol_type = other RNA

SEQ ID NO: 24 - RNA, 24 nt, synthetic construct
  source 1..24: mol_type = other RNA
ctggagttcagacgttgtgctctt

SEQ ID NO: 25 - RNA, 32 nt, synthetic construct; identical to SEQ ID NO: 14
  source 1..32: mol_type = other RNA

SEQ ID NO: 26 - RNA, 24 nt, synthetic construct
  source 1..24: mol_type = other RNA
ctggagttcagaccgtgtgctctt

SEQ ID NO: 27 - RNA, 23 nt, synthetic construct
  source 1..23: mol_type = other RNA
ctggagttcagacgtgttgctct

SEQ ID NO: 28 - RNA, 22 nt, synthetic construct
  source 1..22: mol_type = other RNA
ctgagttcagacgtgttgctct

SEQ ID NO: 29 - RNA, 21 nt, synthetic construct
  source 1..21: mol_type = other RNA
ctgcttcagacgtgttagctt

SEQ ID NO: 30 - RNA, 24 nt, synthetic construct
  source 1..24: mol_type = other RNA
acggagttcagacgtgttgctctt

SEQ ID NO: 31 - RNA, 24 nt, synthetic construct
  source 1..24: mol_type = other RNA
ctggagttcactactgttgctctt

SEQ ID NO: 32 - RNA, 24 nt, synthetic construct
  source 1..24: mol_type = other RNA
ctggagttcagttgtgttgctctt

SEQ ID NO: 33 - RNA, 32 nt, synthetic construct; identical to SEQ ID NO: 3
  source 1..32: mol_type = other RNA

SEQ ID NO: 34 - RNA, 32 nt, synthetic construct; identical to SEQ ID NO: 12
  source 1..32: mol_type = other RNA

SEQ ID NO: 35 - RNA, 24 nt, synthetic construct
  source 1..24: mol_type = other RNA
ctggagttcagacgtgttgctctt

SEQ ID NO: 36 - RNA, 32 nt, synthetic construct; identical to SEQ ID NO: 13
  source 1..32: mol_type = other RNA

SEQ ID NO: 37 - RNA, 24 nt, synthetic construct
  source 1..24: mol_type = other RNA
ctggagttcagacgttgtgctctt

SEQ ID NO: 38 - RNA, 32 nt, synthetic construct; identical to SEQ ID NO: 14
  source 1..32: mol_type = other RNA

SEQ ID NO: 39 - RNA, 24 nt, synthetic construct
  source 1..24: mol_type = other RNA
ctggagttcagaccgtgtgctctt

SEQ ID NO: 40 - RNA, 17 nt, synthetic construct
  source 1..17: mol_type = other RNA
gtacattctagatagcc

SEQ ID NO: 41 - RNA, 17 nt, synthetic construct
  source 1..17: mol_type = other RNA
ggctatctagaatgtac

SEQ ID NO: 42 - RNA, 17 nt, synthetic construct
  source 1..17: mol_type = other RNA
gtacattctagatagcc

SEQ ID NO: 43 - RNA, 17 nt, synthetic construct
  source 1..17: mol_type = other RNA
ggctatctagaatgtac

SEQ ID NO: 44 - RNA, 32 nt, synthetic construct; identical to SEQ ID NO: 3
  source 1..32: mol_type = other RNA

SEQ ID NO: 45 - RNA, 24 nt, synthetic construct
  source 1..24: mol_type = other RNA
ggacatggattcttgtctgtgtcc

SEQ ID NO: 46 - RNA, 24 nt, synthetic construct
  source 1..24: mol_type = other RNA
gatctgtgtcttagacgtgttgcc

SEQ ID NO: 47 - RNA, 32 nt, synthetic construct
  source 1..32: mol_type = other RNA
gatcgtgacgactcttgtctgctgtcctgatc

SEQ ID NO: 48 - RNA, 32 nt, synthetic construct
  source 1..32: mol_type = other RNA
cgtctccagcatgtgtaggtctctgtctctga

SEQ ID NO: 49 - RNA, 21 nt, synthetic construct
  source 1..21: mol_type = other RNA
ggagttcagacgtgttgctct

SEQ ID NO: 50 - RNA, 26 nt, synthetic construct
  source 1..26: mol_type = other RNA
ctggagttcgttgctcttccgatctc

SEQ ID NO: 51 - RNA, 25 nt, synthetic construct
  source 1..25: mol_type = other RNA
ctggacagacgtgtcttccgatctc

SEQ ID NO: 52 - RNA, 32 nt, synthetic construct
  source 1..32: mol_type = other RNA
ctggagttcagatcagacgtgtgtgttgctct

SEQ ID NO: 53 - RNA, 32 nt, synthetic construct
  source 1..32: mol_type = other RNA
ctggagttcagacgtgtagctcgtgtgatctc

SEQ ID NO: 54 - RNA, 32 nt, synthetic construct; identical to SEQ ID NO: 12
  source 1..32: mol_type = other RNA